European Patent Application EP 4 209 226 A1, published July 12, 2023. Title: USE OF POLYPEPTIDE IN DRUG FOR PREVENTING AND TREATING PNEUMONIA. Applicant: ZHEJIANG ECHON BIOMEDICAL CO., LTD. NANNING GENLOCI BIOMEDICAL CO., LTD. Application EP21863250.3. The sequence listing filed with the application follows.

SEQUENCE LISTING (1 sequence)

SEQ ID NO: 1 - protein, 19 aa, Artificial Sequence
  Artificial
MGRFKRFRKKFKKLFKKLS